European Patent Application EP 4 810 054 A1, published September 23, 2026. Title: Agents for Regulating Necroptosis. Applicant: The University of Tokyo. Application JP. The sequence listing filed with the application follows.

SEQUENCE LISTING (8 sequences)

SEQ ID NO: 1 - DNA, 20 bp, synthetic construct
  source 1..20: mol_type = other DNA
gacgccactatgtccatcct

SEQ ID NO: 2 - DNA, 20 bp, synthetic construct
  source 1..20: mol_type = other DNA
tactccagaggccagcagtt

SEQ ID NO: 3 - DNA, 20 bp, synthetic construct
  source 1..20: mol_type = other DNA
caggtccctgtcatgcttct

SEQ ID NO: 4 - DNA, 20 bp, synthetic construct
  source 1..20: mol_type = other DNA
cgttaactgcatctggctga

SEQ ID NO: 5 - DNA, 20 bp, synthetic construct
  source 1..20: mol_type = other DNA
tgttgtgcgaaaagaagtgc

SEQ ID NO: 6 - DNA, 20 bp, synthetic construct
  source 1..20: mol_type = other DNA
tacaaacacagcctcccaca

SEQ ID NO: 7 - DNA, 20 bp, synthetic construct
  source 1..20: mol_type = other DNA
agacctcaacagagccctca

SEQ ID NO: 8 - DNA, 20 bp, synthetic construct
  source 1..20: mol_type = other DNA
ggctggacttttcactctgc